European Patent Application EP 4 772 645 A1, published July 8, 2026. Title: 외래 NAD 의존성 이소시트르산 탈수소효소가 도입된 미생물 및 이를 이용한 L-아미노산 생산 방법. Applicant: 씨제이제일제당 주식회사. The sequence listing filed with the application follows.

SEQUENCE LISTING (86 sequences)

SEQ ID NO: 1 - protein, 393 aa, synthetic construct
MAEKVSFEEGKLQVPDKPVIPYIEGDGVGQDIWKNAQIVFDKAIAKVYGGHKQVIWREVLAGKKAYNETGNWLPNETLEIIKTHLLAIKGPLETPVGGGIRSLNVALRQELDLFACVRPVRYFKGVPSPLKHPEKTAITIFRENTEDIYAGIEWNAGTAEVQKVINFLQDDMQVKKIRFPKSSSIGIKPISIEGSQRLIRAAIEYALANNLTKVTLVHKGNIQKFTEGGFRKWGYELAKREYAAELASGQLVVADIIADNFLQQILLKPERFDVVALTNLNGDYASDALAAQVGGIGISPGANINYQTGHAIFEATHGTAPDIAGQDLANPSSVLLSGCMLFDYIGWSKVSDLIMKAVEKAIANGQVTIDFAKELGVEALTTRQFSEVLLTYL

SEQ ID NO: 2 - DNA, 1182 bp, synthetic construct
  source 1..1182: mol_type = other DNA
atggcagaaaaagtaagttttgaagaaggaaaattacaggtgcctgataagcccatcattccttacattgaaggagatggtgttggtcaggatatttggaagaatgcgcaaatcgtttttgataaagccattgctaaagtttatggaggtcacaagcaggttatttggcgggaggtcttagctggtaaaaaagcttataatgaaacaggcaactggctgcctaatgagactttagaaattatcaagacgcatttacttgctattaaaggtccattggaaactcctgttggaggtggcattcgttccttaaatgttgccctgcgtcaagaattggatctctttgcttgcgtgcggccagtgcgttatttcaaaggtgtccctagtccacttaagcatcctgaaaaaacggctattactatttttcgagaaaatactgaagatatttacgcaggtatcgaatggaatgcgggtacagcagaagttcaaaaggtcatcaactttttacaagatgatatgcgggttaagaaaattcgttttccaaaaagcagcagtatagggattaaacctatttcaattgaaggcagccaacgtttgattcgtgcagctatcgaatatgctctggccaacaatctgaccaaggtaactttggttcataaaggaaatattcaaaaattcactgaaggtggctttagaaaatggggctatgaattagcaaaacgtgagtatgctgccgaacttgccagtggtcaattggtagttgatgatattattgctgacaatttcttgcaacaaattctgctcaagcctgagcattttgatgtagttgccttaacgaatctcaatggggactatgccagcgatgccttagcagcacaagttggcggtattggtatttcgccaggagctaatattaactatcaaacgggacatgctatttttgaagcaacccatggaacggctccagatattgcaggtcaagacttggccaacccatcttctgttttattatcaggctgcatgctttttgactatattggttggtcaaaagtctcagatttaatcatgaaagctgttgaaaaagctattgcaaatggtcaagttaccattgattttgccaaggaactaggggttgaagcattgacaacccgtcagttttctgaagttctattgacttatttatag

SEQ ID NO: 3 - protein, 391 aa, synthetic construct
MAEKIRFESGRLQVPANPVIPYIEGDGVGCDIWKNAKFVFDQAVDKAYKGTRQIEWLEVLAGKKAFDQKDVWLPDATLETIKSHLLAIKGPLETPVGGGIRSLNVTLRQELDLFACVRPVRYFKGVPSPLKNPEKTDITIFRENTEDIYAGIEWEAGTAEVQKVIGFLQDEMQVQKIRFPESSSIGIKPISIEGSKRLIRAAIDYALDKGLSRVTLVHKGNIQKFTEGGFRKWGYELAQEEYAAELASGRLVVDDIIADNFLQQILLKPERFEVVALTNLNGDYASDALAAQVGGIGISPGANINYQTGHAIFEATHGTAPDIAEQDKANPCSLLLSGCMLFDYIGWKEAAELIESALEKSFAAGCFTADLAGDAPSYSTSAFAKVLADNL

SEQ ID NO: 4 - DNA, 1173 bp, synthetic construct
  source 1..1173: mol_type = other DNA
atggcggaaaaaattcgctttgaaagcggccgcctgcaggtgccggcgaacccggtgattccgtatattgaaggcgatggcgtgggctgcgatatttggaaaaacgcgaaatttgtgtttgatcaggcggtggataaagcgtataaaggcacccgccagattgaatggctggaagtgctggcgggcaaaaaagcgtttgatcagaaagatgtgtggctgccggatgcgaccctggaaaccattaaaagccatctgctggcgattaaaggcccgctggaaaccccggtgggcggcggcattcgcagcctgaacgtgaccctgcgccaggaactggatctgtttgcgtgcgtgcgcccggtgcgctattttaaaggcgtgccgagcccgctgaaaaacccggaaaaaaccgatattaccatttttcgcgaaaacaccgaagatatttatgcgggcattgaatgggaagcgggcaccgcggaagtgcagaaagtgattggctttctgcaggatgaaatgcaggtgcagaaaattcgctttccggaaagcagcagcattggcattaaaccgattagcattgaaggcagcaaacgcctgattcgcgcggcgattgattatgcgctggataaaggcctgagccgcgtgaccctggtgcataaaggcaacattcagaaatttaccgaaggcggctttcgcaaatggggctatgaactggcgcaggaagaatatgcggcggaactggcgagcggccgcctggtggtggatgatattattgcggataactttctgcagcagattctgctgaaaccggaacgctttgaagtggtggcgctgaccaacctgaacggcgattatgcgagcgatgcgctggcggcgcaggtgggcggcattggcattagcccgggcgcgaacattaactatcagaccggccatgcgatttttgaagcgacccatggcaccgcgccggatattgcggaacaggataaagcgaacccgtgcagcctgctgctgagcggctgcatgctgtttgattatattggctggaaagaagcggcggaactgattgaaagcgcgctggaaaaaagctttgcggcgggctgctttaccgcggatctggcgggcgatgcgccgagctatagcaccagcgcgtttgcgaaagtgctggcggataacctg

SEQ ID NO: 5 - protein, 396 aa, synthetic construct
MAEKIVLENGQLRVSDHPIIPFIEGDGVGKDIWKSAQSVFDAAVEKAFAGQKKVAWTEVLAGKKSFDQTGSWLPDETVETIKDHLVAIKGPLETPVGGGIRSLNVALRQELDLYACVRPVRYFKGIESPLKHPEKTNITIFRENTEDIYAGIEWEAGSQDVQKIINFLQEDMGVQKIRFPETSSIGIKPISIEGSQRLIRAAIDYALENKLTNVTLVHKGNIQKFTEGGFRKWGYELAQREYAKELASGQLVISDIIADNFLQQILLNPDRFDVVALTNLNGDYASDALAAQVGGIGIAPGANINYRTGHAIFEATHGTAPDIAGQDKANPCSVLLSGCMLFDYIGWTAVSDLITKAIETNFSRGYFTADLAFGKGVEALSTSQFSQRLIDSIGER

SEQ ID NO: 6 - DNA, 1188 bp, synthetic construct
  source 1..1188: mol_type = other DNA
atggcggaaaaaattgtgctggaaaacggccagctgcgcgtgagcgatcatccgattattccgtttattgaaggcgatggcgtgggcaaagatatttggaaaagcgcgcagagcgtgtttgatgcggcggtggaaaaagcgtttgcgggccagaaaaaagtggcgtggaccgaagtgctggcgggcaaaaaaagctttgatcagaccggcagctggctgccggatgaaaccgtggaaaccattaaagatcatctggtggcgattaaaggcccgctggaaaccccggtgggcggcggcattcgcagcctgaacgtggcgctgcgccaggaactggatctgtatgcgtgcgtgcgcccggtgcgctattttaaaggcattgaaagcccgctgaaacatccggaaaaaaccaacattaccatttttcgcgaaaacaccgaagatatttatgcgggcattgaatgggaagcgggcagccaggatgtgcagaaaattattaactttctgcaggaagatatgggcgtgcagaaaattcgctttccggaaaccagcagcattggcattaaaccgattagcattgaaggcagccagcgcctgattcgcgcggcgattgattatgcgctggaaaacaaactgaccaacgtgaccctggtgcataaaggcaacattcagaaatttaccgaaggcggctttcgcaaatggggctatgaactggcgcagcgcgaatatgcgaaagaactggcgagcggccagctggtgattagcgatattattgcggataactttctgcagcagattctgctgaacccggatcgctttgatgtggtggcgctgaccaacctgaacggcgattatgcgagcgatgcgctggcggcgcaggtgggcggcattggcattgcgccgggcgcgaacattaactatcgcaccggccatgcgatttttgaagcgacccatggcaccgcgccggatattgcgggccaggataaagcgaacccgtgcagcgtgctgctgagcggctgcatgctgtttgattatattggctggaccgcggtgagcgatctgattaccaaagcgattgaaaccaactttagccgcggctattttaccgcggatctggcgtttggcaaaggcgtggaagcgctgagcaccagccagtttagccagcgcctgattgatagcattggcgaacgc

SEQ ID NO: 7 - DNA, 40 bp, synthetic construct
  source 1..40: mol_type = other DNA
ttctattgacttatttatagagtctcttcacaaaaagcgc

SEQ ID NO: 8 - DNA, 40 bp, synthetic construct
  source 1..40: mol_type = other DNA
tcgactctagaggatccccggtttgggattcgttgtaatc

SEQ ID NO: 9 - DNA, 36 bp, synthetic construct
  source 1..36: mol_type = other DNA
aattcgagctcggtaccctgctgaatatatgggtgg

SEQ ID NO: 10 - DNA, 36 bp, synthetic construct
  source 1..36: mol_type = other DNA
cttactttttctgccatgagtctccttggttgatgg

SEQ ID NO: 11 - DNA, 42 bp, synthetic construct
  source 1..42: mol_type = other DNA
cccatcaaccaaggagactcatggcagaaaaagtaagttttg

SEQ ID NO: 12 - DNA, 45 bp, synthetic construct
  source 1..45: mol_type = other DNA
agcgctttttgtgaagagactctataaataagtcaatagaacttc

SEQ ID NO: 13 - DNA, 18 bp, synthetic construct
  source 1..18: mol_type = other DNA
cattcgtcgatctctagt

SEQ ID NO: 14 - DNA, 18 bp, synthetic construct
  source 1..18: mol_type = other DNA
caattccttgtcggtgtc

SEQ ID NO: 15 - DNA, 42 bp, synthetic construct
  source 1..42: mol_type = other DNA
cccatcaaccaaggagactcatggcggaaaaaattcgctttg

SEQ ID NO: 16 - DNA, 43 bp, synthetic construct
  source 1..43: mol_type = other DNA
agcgctttttgtgaagagactcaggttatccgccagcactttc

SEQ ID NO: 17 - DNA, 39 bp, synthetic construct
  source 1..39: mol_type = other DNA
cccatcaaccaaggagactcatggcggaaaaaattgtgc

SEQ ID NO: 18 - DNA, 43 bp, synthetic construct
  source 1..43: mol_type = other DNA
agcgctttttgtgaagagactgcgttcgccaatgctatcaatc

SEQ ID NO: 19 - protein, 281 aa, synthetic construct
MLKIAVPNKGSLSERAMEILAEAGYAGRGDSKSLNVFDEANNVEFFFLRPKDIAIYVAGGQLDLGITGRDLARDSQADVHEVLSLGFGSSTFRYAAPADEEWSIEKLDGKRIATSYPNLVRDDLAARGLSAEVLRLDGAVEVSIKLGVADAIADVVSTGRTLRQQGLAPFGEVLCTSEAVIVGRKDEKVTPEQQILLRRIQGILHAQNFLMLDYNVDRDNLDAATAVTPGLSHPQVSPLARDNWVAVRAMVPRRSANAIMDKLAGLGAEAILASEIRIARI

SEQ ID NO: 20 - DNA, 30 bp, synthetic construct
  source 1..30: mol_type = other DNA
gaggagatcaaaacagtgaagacatttgac

SEQ ID NO: 21 - DNA, 30 bp, synthetic construct
  source 1..30: mol_type = other DNA
acaccaagcttgatggatacctctactgca

SEQ ID NO: 22 - DNA, 29 bp, synthetic construct
  source 1..29: mol_type = other DNA
cagtagaggtatccatcaagcttggtgtc

SEQ ID NO: 23 - DNA, 28 bp, synthetic construct
  source 1..28: mol_type = other DNA
actctagaggatccccctagatgcgggc

SEQ ID NO: 24 - DNA, 294 bp, synthetic construct
  source 1..294: mol_type = other DNA
ggcgcttcatgtcaacaatctttaacgttttcaagttcacaagtcgtgttcaaatggtgacaagattggacactgtgctgaattggcaccaagccctcataaatgatagatctaaatcgaatatcaatatatggtctgtttattggaacgcgtcccagtggctgagacgcatccgctaaagccccaggaaccctgtgcagaaagaacaaataatcgtgaattttggcagcaacagcggggcctggtataattgaaaacgtgcaaaagcatagattattggaggagatcaaaaca

SEQ ID NO: 25 - DNA, 30 bp, synthetic construct
  source 1..30: mol_type = other DNA
aagaatgtaccgaggcgcttcatgtcaaca

SEQ ID NO: 26 - DNA, 30 bp, synthetic construct
  source 1..30: mol_type = other DNA
caaatgtcttcactgttttgatctcctcca

SEQ ID NO: 27 - DNA, 19 bp, synthetic construct
  source 1..19: mol_type = other DNA
actgcctggtaccaccaga

SEQ ID NO: 28 - DNA, 20 bp, synthetic construct
  source 1..20: mol_type = other DNA
ctgcctctcacaagttgaag

SEQ ID NO: 29 - DNA, 30 bp, synthetic construct
  source 1..30: mol_type = other DNA
tcgagctcggtacccattggtgctcggcgc

SEQ ID NO: 30 - DNA, 29 bp, synthetic construct
  source 1..29: mol_type = other DNA
tgggatgtttctgtgttgttagtctagtg

SEQ ID NO: 31 - DNA, 34 bp, synthetic construct
  source 1..34: mol_type = other DNA
tcgagctcggtacccaaccaagtttagatgcgcc

SEQ ID NO: 32 - DNA, 31 bp, synthetic construct
  source 1..31: mol_type = other DNA
gctgggatgtttctgccgatagtttatgtca

SEQ ID NO: 33 - DNA, 35 bp, synthetic construct
  source 1..35: mol_type = other DNA
tcgagctcggtacccggtgacagctcgcgccgcat

SEQ ID NO: 34 - DNA, 32 bp, synthetic construct
  source 1..32: mol_type = other DNA
gcgctgggatgtttctggcgaaaagttctccc

SEQ ID NO: 35 - DNA, 33 bp, synthetic construct
  source 1..33: mol_type = other DNA
tcgagctcggtacccttgatgcctgcatgaagg

SEQ ID NO: 36 - DNA, 31 bp, synthetic construct
  source 1..31: mol_type = other DNA
tgacatgaagcgccgaatattgatcctatct

SEQ ID NO: 37 - DNA, 33 bp, synthetic construct
  source 1..33: mol_type = other DNA
ttcgagctcggtacccaccttcagcaaccactc

SEQ ID NO: 38 - DNA, 29 bp, synthetic construct
  source 1..29: mol_type = other DNA
tgacatgaagcgccgaaaaattcttctct

SEQ ID NO: 39 - DNA, 318 bp, synthetic construct
  source 1..318: mol_type = other DNA
agaaacatcccagcgctactaatagggagcgttgaccttccttccacggaccggtaatcggagtgcctaaaaccgcatgcggcttaggctccaagataggttctgcgcggccgggtaatgcatcttctttagcaacaagttgaggggtaggtgcaaataagaacgacatagaaatcgtctcctttctgtttttaatcaacatacaccaccacctaaaaattccccgaccagcaagttcacagtattcgggcacaatatcgttgccaaaatattgtttcggaatatcatgggatacgtacccaacgaaaggaaacactc

SEQ ID NO: 40 - DNA, 32 bp, synthetic construct
  source 1..32: mol_type = other DNA
actagactaacaacacagaaacatcccagcgc

SEQ ID NO: 41 - DNA, 30 bp, synthetic construct
  source 1..30: mol_type = other DNA
tctgcatatttgctcatgagtgtttccttt

SEQ ID NO: 42 - DNA, 33 bp, synthetic construct
  source 1..33: mol_type = other DNA
acataaactatcggcagaaacatcccagcgcta

SEQ ID NO: 43 - DNA, 30 bp, synthetic construct
  source 1..30: mol_type = other DNA
gacagttttggtcatgagtgtttcctttcg

SEQ ID NO: 44 - DNA, 29 bp, synthetic construct
  source 1..29: mol_type = other DNA
aggatcaatattcggcgcttcatgtcaac

SEQ ID NO: 45 - DNA, 30 bp, synthetic construct
  source 1..30: mol_type = other DNA
gaatagtgaaggtcattgttttgatctcct

SEQ ID NO: 46 - DNA, 29 bp, synthetic construct
  source 1..29: mol_type = other DNA
gagaagaatttttcggcgcttcatgtcaa

SEQ ID NO: 47 - DNA, 15 bp, synthetic construct
  source 1..15: mol_type = other DNA
gagcatgcatcaaag

SEQ ID NO: 48 - DNA, 19 bp, synthetic construct
  source 1..19: mol_type = other DNA
agaaatttgatccttataa

SEQ ID NO: 49 - DNA, 17 bp, synthetic construct
  source 1..17: mol_type = other DNA
ttgagagatgcttatcg

SEQ ID NO: 50 - DNA, 20 bp, synthetic construct
  source 1..20: mol_type = other DNA
cacttcagtgcggattccaa

SEQ ID NO: 51 - DNA, 17 bp, synthetic construct
  source 1..17: mol_type = other DNA
agcgggtttaattcagg

SEQ ID NO: 52 - DNA, 18 bp, synthetic construct
  source 1..18: mol_type = other DNA
gtgggtaagggttttcgt

SEQ ID NO: 53 - DNA, 19 bp, synthetic construct
  source 1..19: mol_type = other DNA
cacgaaaatgatcgttttg

SEQ ID NO: 54 - DNA, 18 bp, synthetic construct
  source 1..18: mol_type = other DNA
tatgggattcgatggcca

SEQ ID NO: 55 - DNA, 19 bp, synthetic construct
  source 1..19: mol_type = other DNA
tgtgggaatcgctgggcac

SEQ ID NO: 56 - DNA, 16 bp, synthetic construct
  source 1..16: mol_type = other DNA
cggtcgcccgcatctg

SEQ ID NO: 57 - DNA, 31 bp, synthetic construct
  source 1..31: mol_type = other DNA
ttcgagctcggtacccatgaagtctaccggc

SEQ ID NO: 58 - DNA, 30 bp, synthetic construct
  source 1..30: mol_type = other DNA
gacatgaagcgccgacatctaataaccggg

SEQ ID NO: 59 - DNA, 32 bp, synthetic construct
  source 1..32: mol_type = other DNA
ccgacgaggcctaagaactcattccttctgct

SEQ ID NO: 60 - DNA, 31 bp, synthetic construct
  source 1..31: mol_type = other DNA
ctctagaggatccccttagagtgcattgatc

SEQ ID NO: 61 - DNA, 30 bp, synthetic construct
  source 1..30: mol_type = other DNA
ccggttattagatgtcggcgcttcatgtca

SEQ ID NO: 62 - DNA, 25 bp, synthetic construct
  source 1..25: mol_type = other DNA
ggatgtttctctagatgcgggcgat

SEQ ID NO: 63 - DNA, 29 bp, synthetic construct
  source 1..29: mol_type = other DNA
gcccgcatctagagaaacatcccagcgct

SEQ ID NO: 64 - DNA, 29 bp, synthetic construct
  source 1..29: mol_type = other DNA
agaaggaatgagttcttaggcctcgtcgg

SEQ ID NO: 65 - DNA, 19 bp, synthetic construct
  source 1..19: mol_type = other DNA
ctttcagctttccctcccg

SEQ ID NO: 66 - DNA, 17 bp, synthetic construct
  source 1..17: mol_type = other DNA
gctgtacttttagtaca

SEQ ID NO: 67 - DNA, 37 bp, synthetic construct
  source 1..37: mol_type = other DNA
gaattcgagctcggtacccctcatttttcccaacccc

SEQ ID NO: 68 - DNA, 45 bp, synthetic construct
  source 1..45: mol_type = other DNA
ttcttcaaaacttactttttctgccatgagtctccttggttgatg

SEQ ID NO: 69 - DNA, 40 bp, synthetic construct; identical to SEQ ID NO: 7
  source 1..40: mol_type = other DNA

SEQ ID NO: 70 - DNA, 45 bp, synthetic construct
  source 1..45: mol_type = other DNA
cctgcaggtcgactctagaggatccccttgagttagtccacgccc

SEQ ID NO: 71 - DNA, 34 bp, synthetic construct
  source 1..34: mol_type = other DNA
tcgagctcggtacccaccgaactcctgacagagt

SEQ ID NO: 72 - DNA, 30 bp, synthetic construct
  source 1..30: mol_type = other DNA
acatgaagcgcctcggtacattcttccaca

SEQ ID NO: 73 - DNA, 32 bp, synthetic construct
  source 1..32: mol_type = other DNA
aaaggaaacactcatgagcaaatatgcagacg

SEQ ID NO: 74 - DNA, 27 bp, synthetic construct
  source 1..27: mol_type = other DNA
ctagaggatcccccagccggagaggga

SEQ ID NO: 75 - DNA, 30 bp, synthetic construct
  source 1..30: mol_type = other DNA
aaaggaaacactcatgaccaaaactgtcgc

SEQ ID NO: 76 - DNA, 31 bp, synthetic construct
  source 1..31: mol_type = other DNA
ctagaggatccccacctctggaggcgtggtc

SEQ ID NO: 77 - DNA, 34 bp, synthetic construct
  source 1..34: mol_type = other DNA
cgaaaggaaacactcatgttgaatgtcactgacc

SEQ ID NO: 78 - DNA, 32 bp, synthetic construct
  source 1..32: mol_type = other DNA
ctagaggatccccccgtgctcagcctgaggag

SEQ ID NO: 79 - DNA, 33 bp, synthetic construct
  source 1..33: mol_type = other DNA
ggagatcaaaacaatgaccttcactattcttcc

SEQ ID NO: 80 - DNA, 32 bp, synthetic construct
  source 1..32: mol_type = other DNA
ctagaggatccccacgaaacgtgcacaacctt

SEQ ID NO: 81 - DNA, 27 bp, synthetic construct
  source 1..27: mol_type = other DNA
gagatcaaaacaatgactgtcgcacca

SEQ ID NO: 82 - DNA, 32 bp, synthetic construct
  source 1..32: mol_type = other DNA
ctagaggatccccgggtcgcggccgtagtggc

SEQ ID NO: 83 - DNA, 31 bp, synthetic construct
  source 1..31: mol_type = other DNA
gagaacttttcgccagaaacatcccagcgct

SEQ ID NO: 84 - DNA, 30 bp, synthetic construct
  source 1..30: mol_type = other DNA
agtgacattcaacatgagtgtttcctttcg

SEQ ID NO: 85 - DNA, 29 bp, synthetic construct
  source 1..29: mol_type = other DNA
tggtgcgacagtcattgttttgatctcct

SEQ ID NO: 86 - DNA, 5802 bp, synthetic construct
  source 1..5802: mol_type = other DNA
gttcgcttgctgtccataaaaccgcccagtctagctatcgccatgtaagcccactgcaagctacctgctttctctttgcgcttgcgttttcccttgtccagatagcccagtagctgacattcatccggggtcagcaccgtttctgcggactggctttctacgtgttccgcttcctttagcagcccttgcgccctgagtgcttgcggcagcgtgaagctagcttttatcgccattcgccattcaggctgcgcaactgttgggaagggcgatcggtgcgggcctcttcgctattacgccagctggcgaaagggggatgtgctgcaaggcgattaagttgggtaacgccagggttttcccagtcacgacgttgtaaaacgacggccagtgaattcgagctcggtacccggggatcctctagagtcgacctgcaggcatgcaagcttggcgtaatcatggtcatagctgtttcctgtgtgaaattgttatccgctcacaattccacacaacatacgagccggaagcataaagtgtaaagcctggggtgcctaatgagtgagctaactcacattaattgcgttgcgctcactgcccgctttccagtcgggaaacctgtcgtgccagctgcattaatgaatcggccaacgcgcggggagaggcggtttgcgtattgggcgctcttccgcttcctcgctcactgactcgctgcgctcggtcgttcggctgcggcgagcggtatcagctcactcaaaggcggtaatacggttatccacagaatcaggggataacgcaggaaagaacatgtgagcaaaaggccagcaaaaggccaggaaccgtaaaaaggccgcgttgctggcgtttttccataggctccgcccccctgacgagcatcacaaaaatcgacgctcaagtcagaggtggcgaaacccgacaggactataaagataccaggcgtttccccctggaagctccctcgtgcgctctcctgttccgaccctgccgcttaccggatacctgtccgcctttctcccttcgggaagcgtggcgctttctcaatgctcacgctgtaggtatctcagttcggtgtaggtcgttcgctccaagctgggctgtgtgcacgaaccccccgttcagcccgaccgctgcgccttatccggtaactatcgtcttgagtccaacccggtaagacacgacttatcgccactggcagcagccactggtaacaggattagcagagcgaggtatgtaggcggtgctacagagttcttgaagtggtggcctaactacggctacactagaaggacagtatttggtatctgcgctctgctgaagccagttaccttcggaaaaagagttggtagctcttgatccggcaaacaaaccaccgctggtagcggtggtttttttgtttgcaagcagcagattacgcgcagaaaaaaaggatctcaagaagatcctttgatcttttctacggggtctgacgctcagtggaacgaaaactcacgttaagggattttggtcatgagattatcaaaaaggatcttcacctagatccttttggggtgggcgaagaactccagcatgagatccccgcgctggaggatcatccagccctgatagaaacagaagccactggagcacctcaaaaacaccatcatacactaaatcagtaagttggcagcatcacccgacgcactttgcgccgaataaatacctgtgacggaagatcacttcgcagaataaataaatcctggtgtccctgttgataccgggaagccctgggccaacttttggcgaaaatgagacgttgatcggcacgtaagaggttccaactttcaccataatgaaataagatcactaccgggcgtattttttgagttatcgagattttcaggagctgatagaaacagaagccactggagcacctcaaaaacaccatcatacactaaatcagtaagttggcagcatcacccgacgcactttgcgccgaataaatacctgtgacggaagatcacttcgcagaataaataaatcctggtgtccctgttgataccgggaagccctgggccaacttttggcgaaaatgagacgttgatcggcacgtaagaggttccaactttcaccataatgaaataagatcactaccgggcgtattttttgagttatcgagattttcaggagctctttggcatcgtctctcgcctgtcccctcagttcagtaatttcctgcatttgcctgtttccagtcggtagatattccacaaaacagcagggaagcagcgcttttccgctgcataaccctgcttcggggtcattatagcgattttttcggtatatccatcctttttcgcacgatatacaggattttgccaaagggttcgtgtagactttccttggtgtatccaacggcgtcagccgggcaggataggtgaagtaggcccacccgcgagcgggtgttccttcttcactgtcccttattcgcacctggcggtgctcaacgggaatcctgctctgcgaggctggccggctaccgccggcgtaacagatgagggcaagcggatggctgatgaaaccaagccaaccaggaagggcagcccacctatcaaggtgtactgccttccagacgaacgaagagcgattgaggaaaaggcggcggcggccggcatgagcctgtcggcctacctgctggccgtcggccagggctacaaaatcacgggcgtcgtggactatgagcacgtccgcgagggcgtcccggaaaacgattccgaagcccaacctttcatagaaggcggcggtggaatcgaaatctcgtgatggcaggttgggcgtcgcttggtcggtcatttcgaaaaaggttaggaatacggttagccatttgcctgcttttatatagttcatatgggattcacctttatgttgataagaaataaaagaaaatgccaataggatatcggcattttcttttgcgtttttatttgttaactgttaattgtccttgttcaaggatgctgtctttgacaacagatgttttcttgcctttgatgttcagcaggaagctcggcgcaaacgttgattgtttgtctgcgtagaatcctctgtttgtcatatagcttgtaatcacgacattgtttcctttcgcttgaggtacagcgaagtgtgagtaagtaaaggttacatcgttaggcggatcaagatccatttttaacacaaggccagttttgttcagcggcttgtatgggccagttaaagaattagaaacataaccaagcatgtaaatatcgttagacgtaatgccgtcaatcgtcatttttgatccgcgggagtcagtgaacaggtaccatttgccgttcattttaaagacgttcgcgcgttcaatttcatctgttactgtgttagatgcaatcagcggtttcatcacttttttcagtgtgtaatcatcgtttagctcaatcataccgagagcgccgtttgctaactcagccgtgcgttttttatcgctttgcagaagtttttgactttcttgacggaagaatgatgtgcttttgccatagtatgctttgttaaataaagattcttcgccttggtagccatcttcagttccagtgtttgcttcaaatactaagtatttgtggcctttatcttctacgtagtgaggatctctcagcgtatggttgtcgcctgagctgtagttgccttcatcgatgaactgctgtacattttgatacgtttttccgtcaccgtcaaagattgatttataatcctctacaccgttgatgttcaaagagctgtctgatgctgatacgttaacttgtgcagttgtcagtgtttgtttgccgtaatgtttaccggagaaatcagtgtagaataaacggatttttccgtcagatgtaaatgtggctgaacctgaccattcttgtgtttggtcttttaggatagaatcatttgcatcgaatttgtcgctgtctttaaagacgcggccagcgtttttccagctgtcaatagaagtttcgccgactttttgatagaacatgtaaatcgatgtgtcatccgcatttttaggatctccggctaatgcaaagacgatgtggtagccgtgatagtttgcgacagtgccgtcagcgttttgtaatggccagctgtcccaaacgtccaggccttttgcagaagagatatttttaattgtggacgaatcaaattcagaaacttgatatttttcatttttttgctgttcagggatttgcagcatatcatggcgtgtaatatgggaaatgccgtatgtttccttatatggcttttggttcgtttctttcgcaaacgcttgagttgcgcctcctgccagcagtgcggtagtaaaggttaatactgttgcttgttttgcaaactttttgatgttcatcgttcatgtctccttttttatgtactgtgttagcggtctgcttcttccagccctcctgtttgaagatggcaagttagttacgcacaataaaaaaagacctaaaatatgtaaggggtgacgccaaagtatacactttgccctttacacattttaggtcttgcctgctttatcagtaacaaacccgcgcgatttacttttcgacctcattctattagactctcgtttggattgcaactggtctattttcctcttttgtttgatagaaaatcataaaaggatttgcagactacgggcctaaagaactaaaaaatctatctgtttcttttcattctctgtattttttatagtttctgttgcatgggcataaagttgcctttttaatcacaattcagaaaatatcataatatctcatttcactaaataatagtgaacggcaggtatatgtgatgggttaaaaaggatcaccccagagtcccgctcagaagaactcgtcaagaaggcgatagaaggcgatgcgctgcgaatcgggagcggcgataccgtaaagcacgaggaagcggtcagcccattcgccgccaagctcttcagcaatatcacgggtagccaacgctatgtcctgatagcggtccgccacacccagccggccacagtcgatgaatccagaaaagcggccattttccaccatgatattcggcaagcaggcatcgccatgggtcacgacgagatcctcgccgtcgggcatccgcgccttgagcctggcgaacagttcggctggcgcgagcccctgatgctcttcgtccagatcatcctgatcgacaagaccggcttccatccgagtacgtgctcgctcgatgcgatgtttcgcttggtggtcgaatgggcaggtagccggatcaagcgtatgcagccgccgcattgcatcagccatgatggatactttctcggcaggagcaaggtgagatgacaggagatcctgccccggcacttcgcccaatagcagccagtcccttcccgcttcagtgacaacgtcgagacagctgcgcaaggaacgcccgtcgtggccagccacgatagccgcgctgcctcgtcttggagttcattcagggcaccggacaggtcggtcttgacaaaaagaaccgggcgcccctgcgctgacagccggaacacggcggcatcagagcagccgattgtctgttgtgcccagtcatagccgaatagcctctccacccaagcggccggagaacctgcgtgcaatccatcttgttcaatcatgcgaaacgatcctcatcctgtctcttgatcagatcttgatcccctgcgccatcagatccttggcggcaagaaagccatccagtttactttgcagggcttcccaaccttaccagagggcgccccagctggcaattccg